European Patent Application EP 4 596 584 A1, published August 6, 2025. Title: Trispecific antibodies targeting PD-1, CTLA-4 and VEGF and use thereof. Applicant: HC BIOPHARMA, INC. The sequence listing filed with the application follows.

SEQUENCE LISTING (76 sequences)

SEQ ID NO: 1 - protein, 5 aa, synthetic construct
SYGMS

SEQ ID NO: 2 - protein, 17 aa, synthetic construct
TISGGGRDTYYPDSVKG

SEQ ID NO: 3 - protein, 9 aa, synthetic construct
QNGITWFAD

SEQ ID NO: 4 - protein, 14 aa, synthetic construct
RASESVDNYGISFM

SEQ ID NO: 5 - protein, 7 aa, synthetic construct
AASNQGS

SEQ ID NO: 6 - protein, 9 aa, synthetic construct
QQSKEVPWT

SEQ ID NO: 7 - protein, 118 aa, synthetic construct
EVQLVESGGGLVQPGGSLRLSCAASGFTFSSYGMSWVRQAPGKGLEWVSTISGGGRDTYYPDSVKGRFTISRDNSKNTLYLQMNSLRAEDTAVYYCARQNGITWFADWGQGTLVTVSS

SEQ ID NO: 8 - protein, 111 aa, synthetic construct
DIQMTQSPSSLSASVGDRVTITCRASESVDNYGISFMNWYQQKPGKAPKLLIYAASNQGSGVPSRFSGSGSGTDFTLTISSLQPEDFATYYCQQSKEVPWTFGGGTKVEIK

SEQ ID NO: 9 - protein, 20 aa, synthetic construct
GGGGSGGGGSGGGGSGGGGS

SEQ ID NO: 10 - protein, 249 aa, synthetic construct
EVQLVESGGGLVQPGGSLRLSCAASGFTFSSYGMSWVRQAPGKCLEWVSTISGGGRDTYYPDSVKGRFTISRDNSKNTLYLQMNSLRAEDTAVYYCARQNGITWFADWGQGTLVTVSSGGGGSGGGGSGGGGSGGGGSDIQMTQSPSSLSASVGDRVTITCRASESVDNYGISFMNWYQQKPGKAPKLLIYAASNQGSGVPSRFSGSGSGTDFTLTISSLQPEDFATYYCQQSKEVPWTFGCGTKVEIK

SEQ ID NO: 11 - protein, 115 aa, synthetic construct
EVQLLESGGGLVQPGGSLRLSCAASGSIFSINHMAWYRQAPGKQRELVAGVNSRGTTNYVDSVKGRFTISRDNSKNTLYLQMNSLRAEDTAVYYCRALGGAVAAWGQGTLVTVSS

SEQ ID NO: 12 - protein, 5 aa, synthetic construct
INHMA

SEQ ID NO: 13 - protein, 16 aa, synthetic construct
GVNSRGTTNYVDSVKG

SEQ ID NO: 14 - protein, 7 aa, synthetic construct
LGGAVAA

SEQ ID NO: 15 - protein, 118 aa, synthetic construct
QVQLVESGGGVVQPGRSLRLSCAASGFTFSSYTMHWVRQAPGKGLEWVTFISYDGNNKYYADSVKGRFTISRDNSKNTLYLQMNSLRAEDTAIYYCARTGWLGPFDYWGQGTLVTVSS

SEQ ID NO: 16 - protein, 108 aa, synthetic construct
EIVLTQSPGTLSLSPGERATLSCRASQSVGSSYLAWYQQKPGQAPRLLIYGAFSRATGIPDRFSGSGSGTDFTLTISRLEPEDFAVYYCQQYGSSPWTFGQGTKVEIK

SEQ ID NO: 17 - protein, 5 aa, synthetic construct
SYTMH

SEQ ID NO: 18 - protein, 16 aa, synthetic construct
FISYDGNNKYYADSVK

SEQ ID NO: 19 - protein, 9 aa, synthetic construct
TGWLGPFDY

SEQ ID NO: 20 - protein, 12 aa, synthetic construct
RASQSVGSSYLA

SEQ ID NO: 21 - protein, 7 aa, synthetic construct
GAFSRAT

SEQ ID NO: 22 - protein, 7 aa, synthetic construct
QQYGSSP

SEQ ID NO: 23 - protein, 246 aa, synthetic construct
QVQLVESGGGVVQPGRSLRLSCAASGFTFSSYTMHWVRQAPGKCLEWVTFISYDGNNKYYADSVKGRFTISRDNSKNTLYLQMNSLRAEDTAIYYCARTGWLGPFDYWGQGTLVTVSSGGGGSGGGGSGGGGSGGGGSEIVLTQSPGTLSLSPGERATLSCRASQSVGSSYLAWYQQKPGQAPRLLIYGAFSRATGIPDRFSGSGSGTDFTLTISRLEPEDFAVYYCQQYGSSPWTFGCGTKVEIK

SEQ ID NO: 24 - protein, 123 aa, synthetic construct [sequence omitted]

SEQ ID NO: 25 - protein, 107 aa, synthetic construct [sequence omitted]

SEQ ID NO: 26 - protein, 5 aa, synthetic construct
NYGMN

SEQ ID NO: 27 - protein, 16 aa, synthetic construct
WINTYTGEPTYAADFK

SEQ ID NO: 28 - protein, 14 aa, synthetic construct
YPHYYGSSHWYFDV

SEQ ID NO: 29 - protein, 11 aa, synthetic construct
SASQDISNYLN

SEQ ID NO: 30 - protein, 7 aa, synthetic construct
FTSSLHS

SEQ ID NO: 31 - protein, 7 aa, synthetic construct
QQYSTVP

SEQ ID NO: 32 - protein, 250 aa, synthetic construct
EVQLVESGGGLVQPGGSLRLSCAASGYTFTNYGMNWVRQAPGKCLEWVGWINTYTGEPTYAADFKRRFTFSLDTSKSTAYLQMNSLRAEDTAVYYCAKYPHYYGSSHWYFDVWGQGTLVTVSSGGGGSGGGGSGGGGSGGGGSDIQMTQSPSSLSASVGDRVTITCSASQDISNYLNWYQQKPGKAPKVLIYFTSSLHSGVPSRFSGSGSGTDFTLTISSLQPEDFATYYCQQYSTVPWTFGCGTKVEIK

SEQ ID NO: 33 - protein, 330 aa, synthetic construct [sequence omitted]

SEQ ID NO: 34 - protein, 327 aa, synthetic construct
ASTKGPSVFPLAPCSRSTSESTAALGCLVKDYFPEPVTVSWNSGALTSGVHTFPAVLQSSGLYSLSSVVTVPSSSLGTKTYTCNVDHKPSNTKVDKRVESKYGPPCPPCPAPEFLGGPSVFLFPPKPKDTLMISRTPEVTCVVVDVSQEDPEVQFNWYVDGVEVHNAKTKPREEQFNSTYRVVSVLTVLHQDWLNGKEYKCKVSNKGLPSSIEKTISKAKGQPREPQVYTLPPSQEEMTKNQVSLTCLVKGFYPSDIAVEWESNGQPENNYKTTPPVLDSDGSFFLYSRLTVDKSRWQEGNVFSCSVMHEALHNHYTQKSLSLSLGK

SEQ ID NO: 35 - protein, 327 aa, synthetic construct
ASTKGPSVFPLAPCSRSTSESTAALGCLVKDYFPEPVTVSWNSGALTSGVHTFPAVLQSSGLYSLSSVVTVPSSSLGTKTYTCNVDHKPSNTKVDKRVESKYGPPCPPCPAPEFLGGPSVFLFPPKPKDTLMISRTPEVTCVVVDVSQEDPEVQFNWYVDGVEVHNAKTKPREEQFNSTYRVVSVLTVLHQDWLNGKEYKCKVSNKGLPSSIEKTISKAKGQPREPQVYTLPPSQEEMTKNQVSLTCLVKGFYPSDIAVEWESNGQPENNYKTTPPVLDSDGSFFLYSRLTVDKSRWQEGNVFSCSVMHEALHNHYTQKSLSLSLGA

SEQ ID NO: 36 - protein, 107 aa, synthetic construct [sequence omitted]

SEQ ID NO: 37 - protein, 850 aa, synthetic construct
EVQLVESGGGLVQPGGSLRLSCAASGFTFSSYGMSWVRQAPGKGLEWVSTISGGGRDTYYPDSVKGRFTISRDNSKNTLYLQMNSLRAEDTAVYYCARQNGITWFADWGQGTLVTVSSASTKGPSVFPLAPCSRSTSESTAALGCLVKDYFPEPVTVSWNSGALTSGVHTFPAVLQSSGLYSLSSVVTVPSSSLGTKTYTCNVDHKPSNTKVDKRVESKYGPPCPPCPAPEFLGGPSVFLFPPKPKDTLMISRTPEVTCVVVDVSQEDPEVQFNWYVDGVEVHNAKTKPREEQFNSTYRVVSVLTVLHQDWLNGKEYKCKVSNKGLPSSIEKTISKAKGQPREPQVYTLPPSQEEMTKNQVSLTCLVKGFYPSDIAVEWESNGQPENNYKTTPPVLDSDGSFFLYSRLTVDKSRWQEGNVFSCSVMHEALHNHYTQKSLSLSLGAGGGGSGGGGSGGGGSGGGGSEVQLLESGGGLVQPGGSLRLSCAASGSIFSINHMAWYRQAPGKQRELVAGVNSRGTTNYVDSVKGRFTISRDNSKNTLYLQMNSLRAEDTAVYYCRALGGAVAAWGQGTLVTVSSGGGGSGGGGSGGGGSGGGGSEVQLVESGGGLVQPGGSLRLSCAASGYTFTNYGMNWVRQAPGKCLEWVGWINTYTGEPTYAADFKRRFTFSLDTSKSTAYLQMNSLRAEDTAVYYCAKYPHYYGSSHWYFDVWGQGTLVTVSSGGGGSGGGGSGGGGSGGGGSDIQMTQSPSSLSASVGDRVTITCSASQDISNYLNWYQQKPGKAPKVLIYFTSSLHSGVPSRFSGSGSGTDFTLTISSLQPEDFATYYCQQYSTVPWTFGCGTKVEIK

SEQ ID NO: 38 - protein, 218 aa, synthetic construct
DIQMTQSPSSLSASVGDRVTITCRASESVDNYGISFMNWYQQKPGKAPKLLIYAASNQGSGVPSRFSGSGSGTDFTLTISSLQPEDFATYYCQQSKEVPWTFGGGTKVEIKRTVAAPSVFIFPPSDEQLKSGTASVVCLLNNFYPREAKVQWKVDNALQSGNSQESVTEQDSKDSTYSLSSTLTLSKADYEKHKVYACEVTHQGLSSPVTKSFNRGEC

SEQ ID NO: 39 - protein, 850 aa, synthetic construct
EVQLVESGGGLVQPGGSLRLSCAASGYTFTNYGMNWVRQAPGKCLEWVGWINTYTGEPTYAADFKRRFTFSLDTSKSTAYLQMNSLRAEDTAVYYCAKYPHYYGSSHWYFDVWGQGTLVTVSSGGGGSGGGGSGGGGSGGGGSDIQMTQSPSSLSASVGDRVTITCSASQDISNYLNWYQQKPGKAPKVLIYFTSSLHSGVPSRFSGSGSGTDFTLTISSLQPEDFATYYCQQYSTVPWTFGCGTKVEIKGGGGSGGGGSGGGGSGGGGSEVQLVESGGGLVQPGGSLRLSCAASGFTFSSYGMSWVRQAPGKGLEWVSTISGGGRDTYYPDSVKGRFTISRDNSKNTLYLQMNSLRAEDTAVYYCARQNGITWFADWGQGTLVTVSSASTKGPSVFPLAPCSRSTSESTAALGCLVKDYFPEPVTVSWNSGALTSGVHTFPAVLQSSGLYSLSSVVTVPSSSLGTKTYTCNVDHKPSNTKVDKRVESKYGPPCPPCPAPEFLGGPSVFLFPPKPKDTLMISRTPEVTCVVVDVSQEDPEVQFNWYVDGVEVHNAKTKPREEQFNSTYRVVSVLTVLHQDWLNGKEYKCKVSNKGLPSSIEKTISKAKGQPREPQVYTLPPSQEEMTKNQVSLTCLVKGFYPSDIAVEWESNGQPENNYKTTPPVLDSDGSFFLYSRLTVDKSRWQEGNVFSCSVMHEALHNHYTQKSLSLSLGAGGGGSGGGGSGGGGSGGGGSEVQLLESGGGLVQPGGSLRLSCAASGSIFSINHMAWYRQAPGKQRELVAGVNSRGTTNYVDSVKGRFTISRDNSKNTLYLQMNSLRAEDTAVYYCRALGGAVAAWGQGTLVTVSS

SEQ ID NO: 40 - protein, 218 aa, synthetic construct; identical to SEQ ID NO: 38

SEQ ID NO: 41 - protein, 854 aa, synthetic construct
EVQLVESGGGLVQPGGSLRLSCAASGFTFSSYGMSWVRQAPGKCLEWVSTISGGGRDTYYPDSVKGRFTISRDNSKNTLYLQMNSLRAEDTAVYYCARQNGITWFADWGQGTLVTVSSGGGGSGGGGSGGGGSGGGGSDIQMTQSPSSLSASVGDRVTITCRASESVDNYGISFMNWYQQKPGKAPKLLIYAASNQGSGVPSRFSGSGSGTDFTLTISSLQPEDFATYYCQQSKEVPWTFGCGTKVEIKGGGGSGGGGSGGGGSGGGGSEVQLVESGGGLVQPGGSLRLSCAASGYTFTNYGMNWVRQAPGKGLEWVGWINTYTGEPTYAADFKRRFTFSLDTSKSTAYLQMNSLRAEDTAVYYCAKYPHYYGSSHWYFDVWGQGTLVTVSSASTKGPSVFPLAPCSRSTSESTAALGCLVKDYFPEPVTVSWNSGALTSGVHTFPAVLQSSGLYSLSSVVTVPSSSLGTKTYTCNVDHKPSNTKVDKRVESKYGPPCPPCPAPEFLGGPSVFLFPPKPKDTLMISRTPEVTCVVVDVSQEDPEVQFNWYVDGVEVHNAKTKPREEQFNSTYRVVSVLTVLHQDWLNGKEYKCKVSNKGLPSSIEKTISKAKGQPREPQVYTLPPSQEEMTKNQVSLTCLVKGFYPSDIAVEWESNGQPENNYKTTPPVLDSDGSFFLYSRLTVDKSRWQEGNVFSCSVMHEALHNHYTQKSLSLSLGAGGGGSGGGGSGGGGSGGGGSEVQLLESGGGLVQPGGSLRLSCAASGSIFSINHMAWYRQAPGKQRELVAGVNSRGTTNYVDSVKGRFTISRDNSKNTLYLQMNSLRAEDTAVYYCRALGGAVAAWGQGTLVTVSS

SEQ ID NO: 42 - protein, 214 aa, synthetic construct
DIQMTQSPSSLSASVGDRVTITCSASQDISNYLNWYQQKPGKAPKVLIYFTSSLHSGVPSRFSGSGSGTDFTLTISSLQPEDFATYYCQQYSTVPWTFGQGTKVEIKRTVAAPSVFIFPPSDEQLKSGTASVVCLLNNFYPREAKVQWKVDNALQSGNSQESVTEQDSKDSTYSLSSTLTLSKADYEKHKVYACEVTHQGLSSPVTKSFNRGEC

SEQ ID NO: 43 - protein, 850 aa, synthetic construct
EVQLLESGGGLVQPGGSLRLSCAASGSIFSINHMAWYRQAPGKQRELVAGVNSRGTTNYVDSVKGRFTISRDNSKNTLYLQMNSLRAEDTAVYYCRALGGAVAAWGQGTLVTVSSGGGGSGGGGSGGGGSGGGGSEVQLVESGGGLVQPGGSLRLSCAASGFTFSSYGMSWVRQAPGKGLEWVSTISGGGRDTYYPDSVKGRFTISRDNSKNTLYLQMNSLRAEDTAVYYCARQNGITWFADWGQGTLVTVSSASTKGPSVFPLAPCSRSTSESTAALGCLVKDYFPEPVTVSWNSGALTSGVHTFPAVLQSSGLYSLSSVVTVPSSSLGTKTYTCNVDHKPSNTKVDKRVESKYGPPCPPCPAPEFLGGPSVFLFPPKPKDTLMISRTPEVTCVVVDVSQEDPEVQFNWYVDGVEVHNAKTKPREEQFNSTYRVVSVLTVLHQDWLNGKEYKCKVSNKGLPSSIEKTISKAKGQPREPQVYTLPPSQEEMTKNQVSLTCLVKGFYPSDIAVEWESNGQPENNYKTTPPVLDSDGSFFLYSRLTVDKSRWQEGNVFSCSVMHEALHNHYTQKSLSLSLGAGGGGSGGGGSGGGGSGGGGSEVQLVESGGGLVQPGGSLRLSCAASGYTFTNYGMNWVRQAPGKCLEWVGWINTYTGEPTYAADFKRRFTFSLDTSKSTAYLQMNSLRAEDTAVYYCAKYPHYYGSSHWYFDVWGQGTLVTVSSGGGGSGGGGSGGGGSGGGGSDIQMTQSPSSLSASVGDRVTITCSASQDISNYLNWYQQKPGKAPKVLIYFTSSLHSGVPSRFSGSGSGTDFTLTISSLQPEDFATYYCQQYSTVPWTFGCGTKVEIK

SEQ ID NO: 44 - protein, 218 aa, synthetic construct; identical to SEQ ID NO: 38

SEQ ID NO: 45 - protein, 850 aa, synthetic construct
EVQLVESGGGLVQPGGSLRLSCAASGFTFSSYGMSWVRQAPGKGLEWVSTISGGGRDTYYPDSVKGRFTISRDNSKNTLYLQMNSLRAEDTAVYYCARQNGITWFADWGQGTLVTVSSASTKGPSVFPLAPCSRSTSESTAALGCLVKDYFPEPVTVSWNSGALTSGVHTFPAVLQSSGLYSLSSVVTVPSSSLGTKTYTCNVDHKPSNTKVDKRVESKYGPPCPPCPAPEFLGGPSVFLFPPKPKDTLMISRTPEVTCVVVDVSQEDPEVQFNWYVDGVEVHNAKTKPREEQFNSTYRVVSVLTVLHQDWLNGKEYKCKVSNKGLPSSIEKTISKAKGQPREPQVYTLPPSQEEMTKNQVSLTCLVKGFYPSDIAVEWESNGQPENNYKTTPPVLDSDGSFFLYSRLTVDKSRWQEGNVFSCSVMHEALHNHYTQKSLSLSLGAGGGGSGGGGSGGGGSGGGGSEVQLVESGGGLVQPGGSLRLSCAASGYTFTNYGMNWVRQAPGKCLEWVGWINTYTGEPTYAADFKRRFTFSLDTSKSTAYLQMNSLRAEDTAVYYCAKYPHYYGSSHWYFDVWGQGTLVTVSSGGGGSGGGGSGGGGSGGGGSDIQMTQSPSSLSASVGDRVTITCSASQDISNYLNWYQQKPGKAPKVLIYFTSSLHSGVPSRFSGSGSGTDFTLTISSLQPEDFATYYCQQYSTVPWTFGCGTKVEIKGGGGSGGGGSGGGGSGGGGSEVQLLESGGGLVQPGGSLRLSCAASGSIFSINHMAWYRQAPGKQRELVAGVNSRGTTNYVDSVKGRFTISRDNSKNTLYLQMNSLRAEDTAVYYCRALGGAVAAWGQGTLVTVSS

SEQ ID NO: 46 - protein, 218 aa, synthetic construct; identical to SEQ ID NO: 38

SEQ ID NO: 47 - protein, 715 aa, synthetic construct
EVQLVESGGGLVQPGGSLRLSCAASGFTFSSYGMSWVRQAPGKGLEWVSTISGGGRDTYYPDSVKGRFTISRDNSKNTLYLQMNSLRAEDTAVYYCARQNGITWFADWGQGTLVTVSSASTKGPSVFPLAPCSRSTSESTAALGCLVKDYFPEPVTVSWNSGALTSGVHTFPAVLQSSGLYSLSSVVTVPSSSLGTKTYTCNVDHKPSNTKVDKRVESKYGPPCPPCPAPEFLGGPSVFLFPPKPKDTLMISRTPEVTCVVVDVSQEDPEVQFNWYVDGVEVHNAKTKPREEQFNSTYRVVSVLTVLHQDWLNGKEYKCKVSNKGLPSSIEKTISKAKGQPREPQVYTLPPSQEEMTKNQVSLTCLVKGFYPSDIAVEWESNGQPENNYKTTPPVLDSDGSFFLYSRLTVDKSRWQEGNVFSCSVMHEALHNHYTQKSLSLSLGAGGGGSGGGGSGGGGSGGGGSEVQLVESGGGLVQPGGSLRLSCAASGYTFTNYGMNWVRQAPGKCLEWVGWINTYTGEPTYAADFKRRFTFSLDTSKSTAYLQMNSLRAEDTAVYYCAKYPHYYGSSHWYFDVWGQGTLVTVSSGGGGSGGGGSGGGGSGGGGSDIQMTQSPSSLSASVGDRVTITCSASQDISNYLNWYQQKPGKAPKVLIYFTSSLHSGVPSRFSGSGSGTDFTLTISSLQPEDFATYYCQQYSTVPWTFGCGTKVEIK

SEQ ID NO: 48 - protein, 353 aa, synthetic construct
DIQMTQSPSSLSASVGDRVTITCRASESVDNYGISFMNWYQQKPGKAPKLLIYAASNQGSGVPSRFSGSGSGTDFTLTISSLQPEDFATYYCQQSKEVPWTFGGGTKVEIKRTVAAPSVFIFPPSDEQLKSGTASVVCLLNNFYPREAKVQWKVDNALQSGNSQESVTEQDSKDSTYSLSSTLTLSKADYEKHKVYACEVTHQGLSSPVTKSFNRGECGGGGSGGGGSGGGGSGGGGSEVQLLESGGGLVQPGGSLRLSCAASGSIFSINHMAWYRQAPGKQRELVAGVNSRGTTNYVDSVKGRFTISRDNSKNTLYLQMNSLRAEDTAVYYCRALGGAVAAWGQGTLVTVSS

SEQ ID NO: 49 - protein, 854 aa, synthetic construct
EVQLLESGGGLVQPGGSLRLSCAASGSIFSINHMAWYRQAPGKQRELVAGVNSRGTTNYVDSVKGRFTISRDNSKNTLYLQMNSLRAEDTAVYYCRALGGAVAAWGQGTLVTVSSGGGGSGGGGSGGGGSGGGGSEVQLVESGGGLVQPGGSLRLSCAASGYTFTNYGMNWVRQAPGKGLEWVGWINTYTGEPTYAADFKRRFTFSLDTSKSTAYLQMNSLRAEDTAVYYCAKYPHYYGSSHWYFDVWGQGTLVTVSSASTKGPSVFPLAPCSRSTSESTAALGCLVKDYFPEPVTVSWNSGALTSGVHTFPAVLQSSGLYSLSSVVTVPSSSLGTKTYTCNVDHKPSNTKVDKRVESKYGPPCPPCPAPEFLGGPSVFLFPPKPKDTLMISRTPEVTCVVVDVSQEDPEVQFNWYVDGVEVHNAKTKPREEQFNSTYRVVSVLTVLHQDWLNGKEYKCKVSNKGLPSSIEKTISKAKGQPREPQVYTLPPSQEEMTKNQVSLTCLVKGFYPSDIAVEWESNGQPENNYKTTPPVLDSDGSFFLYSRLTVDKSRWQEGNVFSCSVMHEALHNHYTQKSLSLSLGAGGGGSGGGGSGGGGSGGGGSEVQLVESGGGLVQPGGSLRLSCAASGFTFSSYGMSWVRQAPGKCLEWVSTISGGGRDTYYPDSVKGRFTISRDNSKNTLYLQMNSLRAEDTAVYYCARQNGITWFADWGQGTLVTVSSGGGGSGGGGSGGGGSGGGGSDIQMTQSPSSLSASVGDRVTITCRASESVDNYGISFMNWYQQKPGKAPKLLIYAASNQGSGVPSRFSGSGSGTDFTLTISSLQPEDFATYYCQQSKEVPWTFGCGTKVEIK

SEQ ID NO: 50 - protein, 214 aa, synthetic construct; identical to SEQ ID NO: 42

SEQ ID NO: 51 - protein, 715 aa, synthetic construct
EVQLVESGGGLVQPGGSLRLSCAASGFTFSSYGMSWVRQAPGKGLEWVSTISGGGRDTYYPDSVKGRFTISRDNSKNTLYLQMNSLRAEDTAVYYCARQNGITWFADWGQGTLVTVSSASTKGPSVFPLAPCSRSTSESTAALGCLVKDYFPEPVTVSWNSGALTSGVHTFPAVLQSSGLYSLSSVVTVPSSSLGTKTYTCNVDHKPSNTKVDKRVESKYGPPCPPCPAPEFLGGPSVFLFPPKPKDTLMISRTPEVTCVVVDVSQEDPEVQFNWYVDGVEVHNAKTKPREEQFNSTYRVVSVLTVLHQDWLNGKEYKCKVSNKGLPSSIEKTISKAKGQPREPQVYTLPPCQEEMTKNQVSLWCLVKGFYPSDIAVEWESNGQPENNYKTTPPVLDSDGSFFLYSRLTVDKSRWQEGNVFSCSVMHEALHNHYTQKSLSLSLGAGGGGSGGGGSGGGGSGGGGSEVQLVESGGGLVQPGGSLRLSCAASGYTFTNYGMNWVRQAPGKCLEWVGWINTYTGEPTYAADFKRRFTFSLDTSKSTAYLQMNSLRAEDTAVYYCAKYPHYYGSSHWYFDVWGQGTLVTVSSGGGGSGGGGSGGGGSGGGGSDIQMTQSPSSLSASVGDRVTITCSASQDISNYLNWYQQKPGKAPKVLIYFTSSLHSGVPSRFSGSGSGTDFTLTISSLQPEDFATYYCQQYSTVPWTFGCGTKVEIK

SEQ ID NO: 52 - protein, 218 aa, synthetic construct; identical to SEQ ID NO: 38

SEQ ID NO: 53 - protein, 634 aa, synthetic construct
EVQLLESGGGLVQPGGSLRLSCAASGSIFSINHMAWYRQAPGKQRELVAGVNSRGTTNYVDSVKGRFTISRDNSKNTLYLQMNSLRAEDTAVYYCRALGGAVAAWGQGTLVTVSSGGGGSGGGGSGGGGSGGGGSESKYGPPCPPCPAPEFLGGPSVFLFPPKPKDTLMISRTPEVTCVVVDVSQEDPEVQFNWYVDGVEVHNAKTKPREEQFNSTYRVVSVLTVLHQDWLNGKEYKCKVSNKGLPSSIEKTISKAKGQPREPQVCTLPPSQEEMTKNQVSLSCAVKGFYPSDIAVEWESNGQPENNYKTTPPVLDSDGSFFLVSRLTVDKSRWQEGNVFSCSVMHEALHNRFTQKSLSLSLGAGGGGSGGGGSGGGGSGGGGSEVQLVESGGGLVQPGGSLRLSCAASGYTFTNYGMNWVRQAPGKCLEWVGWINTYTGEPTYAADFKRRFTFSLDTSKSTAYLQMNSLRAEDTAVYYCAKYPHYYGSSHWYFDVWGQGTLVTVSSGGGGSGGGGSGGGGSGGGGSDIQMTQSPSSLSASVGDRVTITCSASQDISNYLNWYQQKPGKAPKVLIYFTSSLHSGVPSRFSGSGSGTDFTLTISSLQPEDFATYYCQQYSTVPWTFGCGTKVEIK

SEQ ID NO: 54 - protein, 768 aa, synthetic construct
EVQLVESGGGLVQPGGSLRLSCAASGFTFSSYGMSWVRQAPGKCLEWVSTISGGGRDTYYPDSVKGRFTISRDNSKNTLYLQMNSLRAEDTAVYYCARQNGITWFADWGQGTLVTVSSGGGGSGGGGSGGGGSGGGGSDIQMTQSPSSLSASVGDRVTITCRASESVDNYGISFMNWYQQKPGKAPKLLIYAASNQGSGVPSRFSGSGSGTDFTLTISSLQPEDFATYYCQQSKEVPWTFGCGTKVEIKGGGGSGGGGSGGGGSGGGGSESKYGPPCPPCPAPEFLGGPSVFLFPPKPKDTLMISRTPEVTCVVVDVSQEDPEVQFNWYVDGVEVHNAKTKPREEQFNSTYRVVSVLTVLHQDWLNGKEYKCKVSNKGLPSSIEKTISKAKGQPREPQVYTLPPCQEEMTKNQVSLWCLVKGFYPSDIAVEWESNGQPENNYKTTPPVLDSDGSFFLYSRLTVDKSRWQEGNVFSCSVMHEALHNHYTQKSLSLSLGAGGGGSGGGGSGGGGSGGGGSEVQLVESGGGLVQPGGSLRLSCAASGYTFTNYGMNWVRQAPGKCLEWVGWINTYTGEPTYAADFKRRFTFSLDTSKSTAYLQMNSLRAEDTAVYYCAKYPHYYGSSHWYFDVWGQGTLVTVSSGGGGSGGGGSGGGGSGGGGSDIQMTQSPSSLSASVGDRVTITCSASQDISNYLNWYQQKPGKAPKVLIYFTSSLHSGVPSRFSGSGSGTDFTLTISSLQPEDFATYYCQQYSTVPWTFGCGTKVEIK

SEQ ID NO: 55 - protein, 634 aa, synthetic construct; identical to SEQ ID NO: 53

SEQ ID NO: 56 - protein, 715 aa, synthetic construct
QVQLVESGGGVVQPGRSLRLSCAASGFTFSSYTMHWVRQAPGKGLEWVTFISYDGNNKYYADSVKGRFTISRDNSKNTLYLQMNSLRAEDTAIYYCARTGWLGPFDYWGQGTLVTVSSASTKGPSVFPLAPCSRSTSESTAALGCLVKDYFPEPVTVSWNSGALTSGVHTFPAVLQSSGLYSLSSVVTVPSSSLGTKTYTCNVDHKPSNTKVDKRVESKYGPPCPPCPAPEFLGGPSVFLFPPKPKDTLMISRTPEVTCVVVDVSQEDPEVQFNWYVDGVEVHNAKTKPREEQFNSTYRVVSVLTVLHQDWLNGKEYKCKVSNKGLPSSIEKTISKAKGQPREPQVYTLPPCQEEMTKNQVSLWCLVKGFYPSDIAVEWESNGQPENNYKTTPPVLDSDGSFFLYSRLTVDKSRWQEGNVFSCSVMHEALHNHYTQKSLSLSLGAGGGGSGGGGSGGGGSGGGGSEVQLVESGGGLVQPGGSLRLSCAASGYTFTNYGMNWVRQAPGKCLEWVGWINTYTGEPTYAADFKRRFTFSLDTSKSTAYLQMNSLRAEDTAVYYCAKYPHYYGSSHWYFDVWGQGTLVTVSSGGGGSGGGGSGGGGSGGGGSDIQMTQSPSSLSASVGDRVTITCSASQDISNYLNWYQQKPGKAPKVLIYFTSSLHSGVPSRFSGSGSGTDFTLTISSLQPEDFATYYCQQYSTVPWTFGCGTKVEIK

SEQ ID NO: 57 - protein, 215 aa, synthetic construct
EIVLTQSPGTLSLSPGERATLSCRASQSVGSSYLAWYQQKPGQAPRLLIYGAFSRATGIPDRFSGSGSGTDFTLTISRLEPEDFAVYYCQQYGSSPWTFGQGTKVEIKRTVAAPSVFIFPPSDEQLKSGTASVVCLLNNFYPREAKVQWKVDNALQSGNSQESVTEQDSKDSTYSLSSTLTLSKADYEKHKVYACEVTHQGLSSPVTKSFNRGEC

SEQ ID NO: 58 - protein, 768 aa, synthetic construct
EVQLVESGGGLVQPGGSLRLSCAASGFTFSSYGMSWVRQAPGKCLEWVSTISGGGRDTYYPDSVKGRFTISRDNSKNTLYLQMNSLRAEDTAVYYCARQNGITWFADWGQGTLVTVSSGGGGSGGGGSGGGGSGGGGSDIQMTQSPSSLSASVGDRVTITCRASESVDNYGISFMNWYQQKPGKAPKLLIYAASNQGSGVPSRFSGSGSGTDFTLTISSLQPEDFATYYCQQSKEVPWTFGCGTKVEIKGGGGSGGGGSGGGGSGGGGSESKYGPPCPPCPAPEFLGGPSVFLFPPKPKDTLMISRTPEVTCVVVDVSQEDPEVQFNWYVDGVEVHNAKTKPREEQFNSTYRVVSVLTVLHQDWLNGKEYKCKVSNKGLPSSIEKTISKAKGQPREPQVCTLPPSQEEMTKNQVSLSCAVKGFYPSDIAVEWESNGQPENNYKTTPPVLDSDGSFFLVSRLTVDKSRWQEGNVFSCSVMHEALHNRFTQKSLSLSLGAGGGGSGGGGSGGGGSGGGGSEVQLVESGGGLVQPGGSLRLSCAASGYTFTNYGMNWVRQAPGKCLEWVGWINTYTGEPTYAADFKRRFTFSLDTSKSTAYLQMNSLRAEDTAVYYCAKYPHYYGSSHWYFDVWGQGTLVTVSSGGGGSGGGGSGGGGSGGGGSDIQMTQSPSSLSASVGDRVTITCSASQDISNYLNWYQQKPGKAPKVLIYFTSSLHSGVPSRFSGSGSGTDFTLTISSLQPEDFATYYCQQYSTVPWTFGCGTKVEIK

SEQ ID NO: 59 - protein, 981 aa, synthetic construct
EVQLVESGGGLVQPGGSLRLSCAASGYTFTNYGMNWVRQAPGKCLEWVGWINTYTGEPTYAADFKRRFTFSLDTSKSTAYLQMNSLRAEDTAVYYCAKYPHYYGSSHWYFDVWGQGTLVTVSSGGGGSGGGGSGGGGSGGGGSDIQMTQSPSSLSASVGDRVTITCSASQDISNYLNWYQQKPGKAPKVLIYFTSSLHSGVPSRFSGSGSGTDFTLTISSLQPEDFATYYCQQYSTVPWTFGCGTKVEIKGGGGSGGGGSGGGGSGGGGSEVQLVESGGGLVQPGGSLRLSCAASGFTFSSYGMSWVRQAPGKGLEWVSTISGGGRDTYYPDSVKGRFTISRDNSKNTLYLQMNSLRAEDTAVYYCARQNGITWFADWGQGTLVTVSSASTKGPSVFPLAPCSRSTSESTAALGCLVKDYFPEPVTVSWNSGALTSGVHTFPAVLQSSGLYSLSSVVTVPSSSLGTKTYTCNVDHKPSNTKVDKRVESKYGPPCPPCPAPEFLGGPSVFLFPPKPKDTLMISRTPEVTCVVVDVSQEDPEVQFNWYVDGVEVHNAKTKPREEQFNSTYRVVSVLTVLHQDWLNGKEYKCKVSNKGLPSSIEKTISKAKGQPREPQVYTLPPSQEEMTKNQVSLTCLVKGFYPSDIAVEWESNGQPENNYKTTPPVLDSDGSFFLYSRLTVDKSRWQEGNVFSCSVMHEALHNHYTQKSLSLSLGAGGGGSGGGGSGGGGSGGGGSQVQLVESGGGVVQPGRSLRLSCAASGFTFSSYTMHWVRQAPGKCLEWVTFISYDGNNKYYADSVKGRFTISRDNSKNTLYLQMNSLRAEDTAIYYCARTGWLGPFDYWGQGTLVTVSSGGGGSGGGGSGGGGSGGGGSEIVLTQSPGTLSLSPGERATLSCRASQSVGSSYLAWYQQKPGQAPRLLIYGAFSRATGIPDRFSGSGSGTDFTLTISRLEPEDFAVYYCQQYGSSPWTFGCGTKVEIK

SEQ ID NO: 60 - protein, 218 aa, synthetic construct; identical to SEQ ID NO: 38

SEQ ID NO: 61 - protein, 985 aa, synthetic construct
EVQLVESGGGLVQPGGSLRLSCAASGFTFSSYGMSWVRQAPGKCLEWVSTISGGGRDTYYPDSVKGRFTISRDNSKNTLYLQMNSLRAEDTAVYYCARQNGITWFADWGQGTLVTVSSGGGGSGGGGSGGGGSGGGGSDIQMTQSPSSLSASVGDRVTITCRASESVDNYGISFMNWYQQKPGKAPKLLIYAASNQGSGVPSRFSGSGSGTDFTLTISSLQPEDFATYYCQQSKEVPWTFGCGTKVEIKGGGGSGGGGSGGGGSGGGGSEVQLVESGGGLVQPGGSLRLSCAASGYTFTNYGMNWVRQAPGKGLEWVGWINTYTGEPTYAADFKRRFTFSLDTSKSTAYLQMNSLRAEDTAVYYCAKYPHYYGSSHWYFDVWGQGTLVTVSSASTKGPSVFPLAPCSRSTSESTAALGCLVKDYFPEPVTVSWNSGALTSGVHTFPAVLQSSGLYSLSSVVTVPSSSLGTKTYTCNVDHKPSNTKVDKRVESKYGPPCPPCPAPEFLGGPSVFLFPPKPKDTLMISRTPEVTCVVVDVSQEDPEVQFNWYVDGVEVHNAKTKPREEQFNSTYRVVSVLTVLHQDWLNGKEYKCKVSNKGLPSSIEKTISKAKGQPREPQVYTLPPSQEEMTKNQVSLTCLVKGFYPSDIAVEWESNGQPENNYKTTPPVLDSDGSFFLYSRLTVDKSRWQEGNVFSCSVMHEALHNHYTQKSLSLSLGAGGGGSGGGGSGGGGSGGGGSQVQLVESGGGVVQPGRSLRLSCAASGFTFSSYTMHWVRQAPGKCLEWVTFISYDGNNKYYADSVKGRFTISRDNSKNTLYLQMNSLRAEDTAIYYCARTGWLGPFDYWGQGTLVTVSSGGGGSGGGGSGGGGSGGGGSEIVLTQSPGTLSLSPGERATLSCRASQSVGSSYLAWYQQKPGQAPRLLIYGAFSRATGIPDRFSGSGSGTDFTLTISRLEPEDFAVYYCQQYGSSPWTFGCGTKVEIK

SEQ ID NO: 62 - protein, 214 aa, synthetic construct; identical to SEQ ID NO: 42

SEQ ID NO: 63 - protein, 984 aa, synthetic construct
EVQLVESGGGLVQPGGSLRLSCAASGFTFSSYGMSWVRQAPGKCLEWVSTISGGGRDTYYPDSVKGRFTISRDNSKNTLYLQMNSLRAEDTAVYYCARQNGITWFADWGQGTLVTVSSGGGGSGGGGSGGGGSGGGGSDIQMTQSPSSLSASVGDRVTITCRASESVDNYGISFMNWYQQKPGKAPKLLIYAASNQGSGVPSRFSGSGSGTDFTLTISSLQPEDFATYYCQQSKEVPWTFGCGTKVEIKGGGGSGGGGSGGGGSGGGGSQVQLVESGGGVVQPGRSLRLSCAASGFTFSSYTMHWVRQAPGKGLEWVTFISYDGNNKYYADSVKGRFTISRDNSKNTLYLQMNSLRAEDTAIYYCARTGWLGPFDYWGQGTLVTVSSASTKGPSVFPLAPCSRSTSESTAALGCLVKDYFPEPVTVSWNSGALTSGVHTFPAVLQSSGLYSLSSVVTVPSSSLGTKTYTCNVDHKPSNTKVDKRVESKYGPPCPPCPAPEFLGGPSVFLFPPKPKDTLMISRTPEVTCVVVDVSQEDPEVQFNWYVDGVEVHNAKTKPREEQFNSTYRVVSVLTVLHQDWLNGKEYKCKVSNKGLPSSIEKTISKAKGQPREPQVYTLPPSQEEMTKNQVSLTCLVKGFYPSDIAVEWESNGQPENNYKTTPPVLDSDGSFFLYSRLTVDKSRWQEGNVFSCSVMHEALHNHYTQKSLSLSLGAGGGGSGGGGSGGGGSGGGGSEVQLVESGGGLVQPGGSLRLSCAASGYTFTNYGMNWVRQAPGKCLEWVGWINTYTGEPTYAADFKRRFTFSLDTSKSTAYLQMNSLRAEDTAVYYCAKYPHYYGSSHWYFDVWGQGTLVTVSSGGGGSGGGGSGGGGSGGGGSDIQMTQSPSSLSASVGDRVTITCSASQDISNYLNWYQQKPGKAPKVLIYFTSSLHSGVPSRFSGSGSGTDFTLTISSLQPEDFATYYCQQYSTVPWTFGCGTKVEIK

SEQ ID NO: 64 - protein, 215 aa, synthetic construct; identical to SEQ ID NO: 57

SEQ ID NO: 65 - protein, 715 aa, synthetic construct; identical to SEQ ID NO: 47

SEQ ID NO: 66 - protein, 353 aa, synthetic construct
EVQLLESGGGLVQPGGSLRLSCAASGSIFSINHMAWYRQAPGKQRELVAGVNSRGTTNYVDSVKGRFTISRDNSKNTLYLQMNSLRAEDTAVYYCRALGGAVAAWGQGTLVTVSSGGGGSGGGGSGGGGSGGGGSDIQMTQSPSSLSASVGDRVTITCRASESVDNYGISFMNWYQQKPGKAPKLLIYAASNQGSGVPSRFSGSGSGTDFTLTISSLQPEDFATYYCQQSKEVPWTFGGGTKVEIKRTVAAPSVFIFPPSDEQLKSGTASVVCLLNNFYPREAKVQWKVDNALQSGNSQESVTEQDSKDSTYSLSSTLTLSKADYEKHKVYACEVTHQGLSSPVTKSFNRGEC

SEQ ID NO: 67 - protein, 719 aa, synthetic construct
EVQLVESGGGLVQPGGSLRLSCAASGYTFTNYGMNWVRQAPGKGLEWVGWINTYTGEPTYAADFKRRFTFSLDTSKSTAYLQMNSLRAEDTAVYYCAKYPHYYGSSHWYFDVWGQGTLVTVSSASTKGPSVFPLAPCSRSTSESTAALGCLVKDYFPEPVTVSWNSGALTSGVHTFPAVLQSSGLYSLSSVVTVPSSSLGTKTYTCNVDHKPSNTKVDKRVESKYGPPCPPCPAPEFLGGPSVFLFPPKPKDTLMISRTPEVTCVVVDVSQEDPEVQFNWYVDGVEVHNAKTKPREEQFNSTYRVVSVLTVLHQDWLNGKEYKCKVSNKGLPSSIEKTISKAKGQPREPQVYTLPPSQEEMTKNQVSLTCLVKGFYPSDIAVEWESNGQPENNYKTTPPVLDSDGSFFLYSRLTVDKSRWQEGNVFSCSVMHEALHNHYTQKSLSLSLGAGGGGSGGGGSGGGGSGGGGSEVQLVESGGGLVQPGGSLRLSCAASGFTFSSYGMSWVRQAPGKCLEWVSTISGGGRDTYYPDSVKGRFTISRDNSKNTLYLQMNSLRAEDTAVYYCARQNGITWFADWGQGTLVTVSSGGGGSGGGGSGGGGSGGGGSDIQMTQSPSSLSASVGDRVTITCRASESVDNYGISFMNWYQQKPGKAPKLLIYAASNQGSGVPSRFSGSGSGTDFTLTISSLQPEDFATYYCQQSKEVPWTFGCGTKVEIK

SEQ ID NO: 68 - protein, 349 aa, synthetic construct
EVQLLESGGGLVQPGGSLRLSCAASGSIFSINHMAWYRQAPGKQRELVAGVNSRGTTNYVDSVKGRFTISRDNSKNTLYLQMNSLRAEDTAVYYCRALGGAVAAWGQGTLVTVSSGGGGSGGGGSGGGGSGGGGSDIQMTQSPSSLSASVGDRVTITCSASQDISNYLNWYQQKPGKAPKVLIYFTSSLHSGVPSRFSGSGSGTDFTLTISSLQPEDFATYYCQQYSTVPWTFGQGTKVEIKRTVAAPSVFIFPPSDEQLKSGTASVVCLLNNFYPREAKVQWKVDNALQSGNSQESVTEQDSKDSTYSLSSTLTLSKADYEKHKVYACEVTHQGLSSPVTKSFNRGEC

SEQ ID NO: 69 - protein, 850 aa, synthetic construct
EVQLLESGGGLVQPGGSLRLSCAASGSIFSINHMAWYRQAPGKQRELVAGVNSRGTTNYVDSVKGRFTISRDNSKNTLYLQMNSLRAEDTAVYYCRALGGAVAAWGQGTLVTVSSGGGGSGGGGSGGGGSGGGGSEVQLVESGGGLVQPGGSLRLSCAASGFTFSSYGMSWVRQAPGKGLEWVSTISGGGRDTYYPDSVKGRFTISRDNSKNTLYLQMNSLRAEDTAVYYCARQNGITWFADWGQGTLVTVSSASTKGPSVFPLAPCSRSTSESTAALGCLVKDYFPEPVTVSWNSGALTSGVHTFPAVLQSSGLYSLSSVVTVPSSSLGTKTYTCNVDHKPSNTKVDKRVESKYGPPCPPCPAPEFLGGPSVFLFPPKPKDTLMISRTPEVTCVVVDVSQEDPEVQFNWYVDGVEVHNAKTKPREEQFNSTYRVVSVLTVLHQDWLNGKEYKCKVSNKGLPSSIEKTISKAKGQPREPQVYTLPPSQEEMTKNQVSLTCLVKGFYPSDIAVEWESNGQPENNYKTTPPVLDSDGSFFLYSRLTVDKSRWQEGNVFSCSVMHEALHNHYTQKSLSLSLGAGGGGSGGGGSGGGGSGGGGSEVQLVESGGGLVQPGGSLRLSCAASGYTFTNYGMNWVRQAPGKGLEWVGWINTYTGEPTYAADFKRRFTFSLDTSKSTAYLQMNSLRAEDTAVYYCAKYPHYYGSSHWYFDVWGQGTLVTVSSGGGGSGGGGSGGGGSGGGGSDIQMTQSPSSLSASVGDRVTITCSASQDISNYLNWYQQKPGKAPKVLIYFTSSLHSGVPSRFSGSGSGTDFTLTISSLQPEDFATYYCQQYSTVPWTFGQGTKVEIK

SEQ ID NO: 70 - protein, 218 aa, synthetic construct; identical to SEQ ID NO: 38

SEQ ID NO: 71 - protein, 854 aa, synthetic construct
EVQLVESGGGLVQPGGSLRLSCAASGYTFTNYGMNWVRQAPGKGLEWVGWINTYTGEPTYAADFKRRFTFSLDTSKSTAYLQMNSLRAEDTAVYYCAKYPHYYGSSHWYFDVWGQGTLVTVSSASTKGPSVFPLAPCSRSTSESTAALGCLVKDYFPEPVTVSWNSGALTSGVHTFPAVLQSSGLYSLSSVVTVPSSSLGTKTYTCNVDHKPSNTKVDKRVESKYGPPCPPCPAPEFLGGPSVFLFPPKPKDTLMISRTPEVTCVVVDVSQEDPEVQFNWYVDGVEVHNAKTKPREEQFNSTYRVVSVLTVLHQDWLNGKEYKCKVSNKGLPSSIEKTISKAKGQPREPQVYTLPPSQEEMTKNQVSLTCLVKGFYPSDIAVEWESNGQPENNYKTTPPVLDSDGSFFLYSRLTVDKSRWQEGNVFSCSVMHEALHNHYTQKSLSLSLGAGGGGSGGGGSGGGGSGGGGSEVQLLESGGGLVQPGGSLRLSCAASGSIFSINHMAWYRQAPGKQRELVAGVNSRGTTNYVDSVKGRFTISRDNSKNTLYLQMNSLRAEDTAVYYCRALGGAVAAWGQGTLVTVSSGGGGSGGGGSGGGGSGGGGSEVQLVESGGGLVQPGGSLRLSCAASGFTFSSYGMSWVRQAPGKCLEWVSTISGGGRDTYYPDSVKGRFTISRDNSKNTLYLQMNSLRAEDTAVYYCARQNGITWFADWGQGTLVTVSSGGGGSGGGGSGGGGSGGGGSDIQMTQSPSSLSASVGDRVTITCRASESVDNYGISFMNWYQQKPGKAPKLLIYAASNQGSGVPSRFSGSGSGTDFTLTISSLQPEDFATYYCQQSKEVPWTFGCGTKVEIK

SEQ ID NO: 72 - protein, 214 aa, synthetic construct; identical to SEQ ID NO: 42

SEQ ID NO: 73 - protein, 854 aa, synthetic construct
EVQLVESGGGLVQPGGSLRLSCAASGFTFSSYGMSWVRQAPGKCLEWVSTISGGGRDTYYPDSVKGRFTISRDNSKNTLYLQMNSLRAEDTAVYYCARQNGITWFADWGQGTLVTVSSGGGGSGGGGSGGGGSGGGGSDIQMTQSPSSLSASVGDRVTITCRASESVDNYGISFMNWYQQKPGKAPKLLIYAASNQGSGVPSRFSGSGSGTDFTLTISSLQPEDFATYYCQQSKEVPWTFGCGTKVEIKGGGGSGGGGSGGGGSGGGGSEVQLLESGGGLVQPGGSLRLSCAASGSIFSINHMAWYRQAPGKQRELVAGVNSRGTTNYVDSVKGRFTISRDNSKNTLYLQMNSLRAEDTAVYYCRALGGAVAAWGQGTLVTVSSGGGGSGGGGSGGGGSGGGGSEVQLVESGGGLVQPGGSLRLSCAASGYTFTNYGMNWVRQAPGKGLEWVGWINTYTGEPTYAADFKRRFTFSLDTSKSTAYLQMNSLRAEDTAVYYCAKYPHYYGSSHWYFDVWGQGTLVTVSSASTKGPSVFPLAPCSRSTSESTAALGCLVKDYFPEPVTVSWNSGALTSGVHTFPAVLQSSGLYSLSSVVTVPSSSLGTKTYTCNVDHKPSNTKVDKRVESKYGPPCPPCPAPEFLGGPSVFLFPPKPKDTLMISRTPEVTCVVVDVSQEDPEVQFNWYVDGVEVHNAKTKPREEQFNSTYRVVSVLTVLHQDWLNGKEYKCKVSNKGLPSSIEKTISKAKGQPREPQVYTLPPSQEEMTKNQVSLTCLVKGFYPSDIAVEWESNGQPENNYKTTPPVLDSDGSFFLYSRLTVDKSRWQEGNVFSCSVMHEALHNHYTQKSLSLSLGA

SEQ ID NO: 74 - protein, 214 aa, synthetic construct; identical to SEQ ID NO: 42

SEQ ID NO: 75 - protein, 854 aa, synthetic construct
EVQLVESGGGLVQPGGSLRLSCAASGYTFTNYGMNWVRQAPGKGLEWVGWINTYTGEPTYAADFKRRFTFSLDTSKSTAYLQMNSLRAEDTAVYYCAKYPHYYGSSHWYFDVWGQGTLVTVSSASTKGPSVFPLAPCSRSTSESTAALGCLVKDYFPEPVTVSWNSGALTSGVHTFPAVLQSSGLYSLSSVVTVPSSSLGTKTYTCNVDHKPSNTKVDKRVESKYGPPCPPCPAPEFLGGPSVFLFPPKPKDTLMISRTPEVTCVVVDVSQEDPEVQFNWYVDGVEVHNAKTKPREEQFNSTYRVVSVLTVLHQDWLNGKEYKCKVSNKGLPSSIEKTISKAKGQPREPQVYTLPPSQEEMTKNQVSLTCLVKGFYPSDIAVEWESNGQPENNYKTTPPVLDSDGSFFLYSRLTVDKSRWQEGNVFSCSVMHEALHNHYTQKSLSLSLGAGGGGSGGGGSGGGGSGGGGSEVQLVESGGGLVQPGGSLRLSCAASGFTFSSYGMSWVRQAPGKCLEWVSTISGGGRDTYYPDSVKGRFTISRDNSKNTLYLQMNSLRAEDTAVYYCARQNGITWFADWGQGTLVTVSSGGGGSGGGGSGGGGSGGGGSDIQMTQSPSSLSASVGDRVTITCRASESVDNYGISFMNWYQQKPGKAPKLLIYAASNQGSGVPSRFSGSGSGTDFTLTISSLQPEDFATYYCQQSKEVPWTFGCGTKVEIKGGGGSGGGGSGGGGSGGGGSEVQLLESGGGLVQPGGSLRLSCAASGSIFSINHMAWYRQAPGKQRELVAGVNSRGTTNYVDSVKGRFTISRDNSKNTLYLQMNSLRAEDTAVYYCRALGGAVAAWGQGTLVTVSS

SEQ ID NO: 76 - protein, 214 aa, synthetic construct; identical to SEQ ID NO: 42